European Patent Application EP 4 512 830 A2, published February 26, 2025. Title: Antibodies useful in cancer diagnosis. Applicant: Astellas Pharma Inc. The sequence listing filed with the application follows.

SEQUENCE LISTING (61 sequences)

SEQ ID NO: 1 - protein, 220 aa, Homo sapiens
MASAGMQILGVVLTLLGWVNGLVSCALPMWKVTAFIGNSIVVAQVVWEGLWMSCVVQSTGQMQCKVYDSLLALPQDLQAARALCVIALLVALFGLLVYLAGAKCTTCVEEKDSKARLVLTSGIVFVISGVLTLIPVCWTAHAIIRDFYNPLVAEAQKRELGASLYLGWAASGLLLLGGGLLCCTCPSGGSQGPSHYMARYSTSAPAISRGPSEYPTKNYV

SEQ ID NO: 2 - protein, 217 aa, Homo sapiens
MASTGLELLGMTLAVLGWLGTLVSCALPLWKVTAFIGNSIVVAQVVWEGLWMSCVVQSTGQMQCKVYDSLLALPQDLQAARALCVIALLLALLGLLVAITGAQCTTCVEDEGAKARIVLTAGVILLLAGILVLIPVCWTAHAIIQDFYNPLVAEALKRELGASLYLGWAAAALLMLGGGLLCCTCPPPQVERPRGPRLGYSIPSRSGASGLDKRDYV

SEQ ID NO: 3 - protein, 220 aa, Homo sapiens
MSMGLEITGTALAVLGWLGTIVCCALPMWRVSAFIGSNIITSQNIWEGLWMNCVVQSTGQMQCKVYDSLLALPQDLQAARALIVVAILLAAFGLLVALVGAQCTNCVQDDTAKAKITIVAGVLFLLAALLTLVPVSWSANTIIRDFYNPVVPEAQKREMGAGLYVGWAAAALQLLGGALLCCSCPPREKKYTATKVVYSAPRSTGPGASLGTGYDRKDYV

SEQ ID NO: 4 - protein, 209 aa, Homo sapiens
MASMGLQVMGIALAVLGWLAVMLCCALPMWRVTAFIGSNIVTSQTIWEGLWMNCVVQSTGQMQCKVYDSLLALPQDLQAARALVIISIIVAALGVLLSVVGGKCTNCLEDESAKAKTMIVAGVVFLLAGLMVIVPVSWTAHNIIQDFYNPLVASGQKREMGASLYVGWAASGLLLLGGGLLCCNCPPRTDKPYSAKYSAARSAAASNYV

SEQ ID NO: 5 - protein, 219 aa, Mus musculus
MASTGLQILGIVLTLLGWVNALVSCALPMWKVTAFIGNSIVVAQMVWEGLWMSCVVQSTGQMQCKVYDSLLALPQDLQAARALCVVTLLIVLLGLLVYLAGAKCTTCVEDRNSKSRLVLISGIIFVISGVLTLIPVCWTAHSIIQDFYNPLVADAQKRELGASLYLGWAASGLLLLGGGLLCCACSSGGTQGPRHYMACYSTSVPHSRGPSEYPTKNYV

SEQ ID NO: 6 - protein, 41 aa, synthetic construct
  REGION 1..41: note = Peptide
LLCCTCPSGGSQGPSHYMARYSTSAPAISRGPSEYPTKNYV

SEQ ID NO: 7 - protein, 40 aa, synthetic construct
  REGION 1..40: note = Peptide
LLCCACSSGGTQGPRHYMACYSTSVPHSRGPSEYPTKNYV

SEQ ID NO: 8 - protein, 38 aa, synthetic construct
  REGION 1..38: note = Peptide
CTCPSGGSQGPSHYMARYSTSAPAISRGPSEYPTKNYV

SEQ ID NO: 9 - protein, 14 aa, synthetic construct
  REGION 1..14: note = Peptide
CTCPSGGSQGPSHY

SEQ ID NO: 10 - protein, 15 aa, synthetic construct
  REGION 1..15: note = Peptide
PSGGSQGPSHYMARY

SEQ ID NO: 11 - protein, 15 aa, synthetic construct
  REGION 1..15: note = Peptide
SQGPSHYMARYSTSA

SEQ ID NO: 12 - protein, 15 aa, synthetic construct
  REGION 1..15: note = Peptide
SHYMARYSTSAPAIS

SEQ ID NO: 13 - protein, 15 aa, synthetic construct
  REGION 1..15: note = Peptide
ARYSTSAPAISRGPS

SEQ ID NO: 14 - protein, 15 aa, synthetic construct
  REGION 1..15: note = Peptide
TSAPAISRGPSEYPT

SEQ ID NO: 15 - protein, 15 aa, synthetic construct
  REGION 1..15: note = Peptide
AISRGPSEYPTKNYV

SEQ ID NO: 16 - protein, 15 aa, synthetic construct
  REGION 1..15: note = Peptide
YMARYSTSAPAISRG

SEQ ID NO: 17 - protein, 15 aa, synthetic construct
  REGION 1..15: note = Peptide
RYSTSAPAISRGPSE

SEQ ID NO: 18 - protein, 15 aa, synthetic construct
  REGION 1..15: note = Peptide
YSTSAPAISRGPSEY

SEQ ID NO: 19 - protein, 15 aa, synthetic construct
  REGION 1..15: note = Peptide
STSAPAISRGPSEYP

SEQ ID NO: 20 - protein, 15 aa, synthetic construct
  REGION 1..15: note = Peptide
SAPAISRGPSEYPTK

SEQ ID NO: 21 - protein, 15 aa, synthetic construct
  REGION 1..15: note = Peptide
APAISRGPSEYPTKN

SEQ ID NO: 22 - protein, 15 aa, synthetic construct
  REGION 1..15: note = Peptide
PAISRGPSEYPTKNY

SEQ ID NO: 23 - protein, 14 aa, synthetic construct
  REGION 1..14: note = Peptide
ISRGPSEYPTKNYV

SEQ ID NO: 24 - protein, 13 aa, synthetic construct
  REGION 1..13: note = Peptide
SRGPSEYPTKNYV

SEQ ID NO: 25 - protein, 12 aa, synthetic construct
  REGION 1..12: note = Peptide
RGPSEYPTKNYV

SEQ ID NO: 26 - protein, 11 aa, synthetic construct
  REGION 1..11: note = Peptide
GPSEYPTKNYV

SEQ ID NO: 27 - protein, 10 aa, synthetic construct
  REGION 1..10: note = Peptide
PSEYPTKNYV

SEQ ID NO: 28 - protein, 9 aa, synthetic construct
  REGION 1..9: note = Peptide
SEYPTKNYV

SEQ ID NO: 29 - protein, 8 aa, synthetic construct
  REGION 1..8: note = Peptide
EYPTKNYV

SEQ ID NO: 30 - protein, 7 aa, synthetic construct
  REGION 1..7: note = Peptide
YPTKNYV

SEQ ID NO: 31 - protein, 6 aa, synthetic construct
  REGION 1..6: note = Peptide
PTKNYV

SEQ ID NO: 32 - protein, 5 aa, synthetic construct
  REGION 1..5: note = Peptide
PTKNY

SEQ ID NO: 33 - protein, 4 aa, synthetic construct
  REGION 1..4: note = Peptide
PTKN

SEQ ID NO: 34 - protein, 40 aa, synthetic construct
  REGION 1..40: note = Peptide
LCCTCPSGGSQGPSHYMARYSTSAPAISRGPSEYPTKNYV

SEQ ID NO: 35 - protein, 37 aa, synthetic construct
  REGION 1..37: note = Peptide
LCCTCPPPQVERPRGPRLGYSIPSRSGASGLDKRDYV

SEQ ID NO: 36 - protein, 41 aa, synthetic construct
  REGION 1..41: note = Peptide
LCCSCPPREKKYTATKVVYSAPRSTGPGASLGTGYDRKDYV

SEQ ID NO: 37 - protein, 29 aa, synthetic construct
  REGION 1..29: note = Peptide
LCCNCPPRTDKPYSAKYSAARSAAASNYV

SEQ ID NO: 38 - protein, 7 aa, synthetic construct
  REGION 1..7: note = Peptide
EYPTKNY

SEQ ID NO: 39 - protein, 4 aa, synthetic construct
  REGION 1..4: note = Peptide
RGPS

SEQ ID NO: 40 - protein, 114 aa, synthetic construct
  REGION 1..114: note = Antibody chain
EVQLQQSGTVLARPGASVRMSCRTSGYIFTTYWIHWVKERPGQGLVWIGAIFPGNSDTTYNQKFRGKASLTAVTSASTAYLDLSSLTDEDSAVYYCTREFYATWGQGTTLTVSS

SEQ ID NO: 41 - protein, 112 aa, synthetic construct
  REGION 1..112: note = Antibody chain
DIVLTQNPLTLSVTIGQTASISCKSSQNLLYSDGKTYLNWLLQRPGQSPKRLIYLMSKLDSGVPDRFTGSGSGTDFTLKISRVEAEDLGVYYCWQGTHFPWTFGGGTKLENT

SEQ ID NO: 42 - protein, 114 aa, synthetic construct
  REGION 1..114: note = Antibody chain
EVQLQQSGTVLARPGASVKMSCRTSGYTFTTYWMHWVRERPGQGLEWIGAIYPENSDATYNQKFKGKASLTAVTSASTAYLELSSLTDEDSAVYYCTREFYATWGQGTTLTVSS

SEQ ID NO: 43 - protein, 112 aa, synthetic construct
  REGION 1..112: note = Antibody chain
DVVMTQNPLTLSVTIGQTASISCKSSQNLLYSDGKTYLNWLLQRPGQSPKRLIYLMSKLDSGVPDRFTGSGSRTDFTLKISRVEAEDLGVYYCWQGTHFPWTFGGGTKLEIT

SEQ ID NO: 44 - protein, 114 aa, synthetic construct; identical to SEQ ID NO: 42
  REGION 1..114: note = Antibody chain

SEQ ID NO: 45 - protein, 112 aa, synthetic construct
  REGION 1..112: note = Antibody chain
DIVLTQNPLTLSVTIGQTASISCKSSQNLLYSDGKTYLNWLLQRPGQSPKRLIYLMSKLESGVPDRFTGSGSGTEFTLKISRVEAEDLGVYYCWQGTHFPWTFGGGTKLEIS

SEQ ID NO: 46 - protein, 17 aa, synthetic construct
  REGION 1..17: note = Peptide
CRDFYNPLVAEAQKREL

SEQ ID NO: 47 - protein, 20 aa, synthetic construct
  REGION 1..20: note = Peptide
GGGLLCCTCPSGGSQGPSHY

SEQ ID NO: 48 - protein, 21 aa, synthetic construct
  REGION 1..21: note = Peptide
CARYSTSAPAISRGPSEYPTK

SEQ ID NO: 49 - protein, 39 aa, synthetic construct
  REGION 1..39: note = Peptide
CCTCPSGGSQGPSHYMARYSTSAPAISRGPSEYPTKNYV

SEQ ID NO: 50 - protein, 61 aa, synthetic construct
  REGION 1..61: note = Peptide
AKCTTCVEEKDSKARLVLTSGIVFVISGVLTLIPVCWTAHAIIRDFYNPLVAEAQKRELGA

SEQ ID NO: 51 - protein, 8 aa, synthetic construct
  REGION 1..8: note = Variable heavy chain CDR
GYIFTTYW

SEQ ID NO: 52 - protein, 8 aa, synthetic construct
  REGION 1..8: note = Variable heavy chain CDR
IFPGNSDT

SEQ ID NO: 53 - protein, 7 aa, synthetic construct
  REGION 1..7: note = Variable heavy chain CDR
TREFYAT

SEQ ID NO: 54 - protein, 11 aa, synthetic construct
  REGION 1..11: note = Variable light chain CDR
QNLLYSDGKTY

SEQ ID NO: 55 - skipped

SEQ ID NO: 56 - protein, 9 aa, synthetic construct
  REGION 1..9: note = Variable light chain CDR
WQGTHFPWT

SEQ ID NO: 57 - protein, 8 aa, synthetic construct
  REGION 1..8: note = Variable heavy chain CDR
GYTFTTYW

SEQ ID NO: 58 - protein, 8 aa, synthetic construct
  REGION 1..8: note = Variable heavy chain CDR
IYPENSDA

SEQ ID NO: 59 - protein, 5 aa, synthetic construct
  REGION 1..5: note = Peptide
EYPTK

SEQ ID NO: 60 - protein, 6 aa, synthetic construct
  REGION 1..6: note = Peptide
EYPTKN

SEQ ID NO: 61 - protein, 6 aa, synthetic construct
  REGION 1..6: note = Peptide
YPTKNY